European Patent Specification EP 3 494 791 B1, published March 1, 2023. Title: TREATMENT OF DISEASE WITH POLY-N-ACETYLGLUCOSAMINE NANOFIBERS. Applicant: Marine Polymer Technologies, Inc. Application EP 18199627.3. The sequence listing filed with the application follows.

SEQUENCE LISTING (6 sequences)

SEQ ID NO: 1 - DNA, 19 bp, Artificial Sequence
  Collagen I forward primer for RT-PCR
acggctgcacgagtcacac

SEQ ID NO: 2 - DNA, 17 bp, Artificial Sequence
  Collagen I reverse primer for RT-PCR
ggcaggcgggaggtctt

SEQ ID NO: 3 - DNA, 28 bp, Artificial Sequence
  Collagen III forward primer for RT-PCR
gttctagaggatggctgtactaaacaca

SEQ ID NO: 4 - DNA, 22 bp, Artificial Sequence
  Collagen III reverse primer for RT-PCR
ttgccttgcgtgtttgatattc

SEQ ID NO: 5 - DNA, 24 bp, Artificial Sequence
  HPRT forward primer for RT-PCR
aaggacctctcgaagtgttggata

SEQ ID NO: 6 - DNA, 25 bp, Artificial Sequence
  HPRT reverse primer for RT-PCR
catttaaaaggaactgttgacaacg